European Patent Application EP 4 218 825 A1, published August 2, 2023. Title: A conjugates of a functional polypeptide variant and uses thereof. Applicant: PROABTECH INC. The sequence listing filed with the application follows.

SEQUENCE LISTING (113 sequences)

SEQ ID NO: 1 - protein, 31 aa, Artificial Sequence
  GLP1 variant
  MISC_FEATURE (1)..(31): This sequence is represented by following in this application. His-X2-X3-X4-X5-Phe-Thr-Ser-X9-X10-X11-X12-X13-Leu-X15-X16-Gln-Ala-Ala-X20-X21-X22-ile-X24-X25-Leu-X27-X28-Gly-Arg-X31
HXXXXFTSXXXXXLXXQAAXXXIXXLXXGRX

SEQ ID NO: 2 - protein, 31 aa, Artificial Sequence
  GLP1 variant
  MISC_FEATURE (1)..(31): X is unnatural amino acid comprising tetrazine group or its variant, or triazine group or its variant.
HGEGTFTSDVSSYLEGQAAKEFIAWLVKGRX

SEQ ID NO: 3 - protein, 31 aa, Artificial Sequence
  GLP1 variant
  MISC_FEATURE (1)..(31): X is unnatural amino acid comprising tetrazine group or its variant, or triazine group or its variant.
HGEGTFTSDXSSYLEGQAAKEFIAWLVKGRG

SEQ ID NO: 4 - protein, 31 aa, Artificial Sequence
  GLP1 variant
  MISC_FEATURE (1)..(31): X is unnatural amino acid comprising tetrazine group or its variant, or triazine group or its variant.
HGEGTFTSDVSSXLEGQAAKEFIAWLVKGRG

SEQ ID NO: 5 - protein, 31 aa, Artificial Sequence
  GLP1 variant
  MISC_FEATURE (1)..(31): X is unnatural amino acid comprising tetrazine group or its variant, or triazine group or its variant.
HGEGTFTSDVSSYLEGQAAKEXIAWLVKGRG

SEQ ID NO: 6 - protein, 31 aa, Artificial Sequence
  GLP1 variant
  MISC_FEATURE (1)..(31): X is unnatural amino acid comprising tetrazine group or its variant, or triazine group or its variant.
HGEGTFTSDVSSYLEGQAAKEFIAWLVRGRX

SEQ ID NO: 7 - protein, 31 aa, Artificial Sequence
  GLP1 variant
  MISC_FEATURE (1)..(31): X is unnatural amino acid comprising tetrazine group or its variant, or triazine group or its variant.
HAEGTFTSDXSSYLEGQAAKEFIAWLVRGRG

SEQ ID NO: 8 - protein, 31 aa, Artificial Sequence
  GLP1 variant
  MISC_FEATURE (1)..(31): X is unnatural amino acid comprising tetrazine group or its variant, or triazine group or its variant.
HAEGTFTSDVSSXLEGQAAKEFIAWLVRGRG

SEQ ID NO: 9 - protein, 31 aa, Artificial Sequence
  GLP1 variant
  MISC_FEATURE (1)..(31): X is unnatural amino acid comprising tetrazine group or its variant, or triazine group or its variant.
HAEGTFTSDVSSYLEGQAAKEXIAWLVRGRG

SEQ ID NO: 10 - protein, 31 aa, Artificial Sequence
  GLP1 variant
  MISC_FEATURE (1)..(31): X is unnatural amino acid comprising tetrazine group or its variant, or triazine group or its variant.
HGEGTFTSDXSSYLEGQAAKEFIAWLVRGRG

SEQ ID NO: 11 - protein, 31 aa, Artificial Sequence
  GLP1 variant
  MISC_FEATURE (1)..(31): X is unnatural amino acid comprising tetrazine group or its variant, or triazine group or its variant.
HGEGTFTSDVSSXLEGQAAKEFIAWLVRGRG

SEQ ID NO: 12 - protein, 31 aa, Artificial Sequence
  GLP1 variant
  MISC_FEATURE (1)..(31): X is unnatural amino acid comprising tetrazine group or its variant, or triazine group or its variant.
HGEGTFTSDVSSYLEGQAAKEXIAWLVRGRG

SEQ ID NO: 13 - protein, 31 aa, Artificial Sequence
  GLP1 variant
  MISC_FEATURE (1)..(31): X is unnatural amino acid comprising tetrazine group or its variant, or triazine group or its variant.
HGEGTFTSDXSSYLEGQAAKEFIAWLVKGRX

SEQ ID NO: 14 - protein, 31 aa, Artificial Sequence
  GLP1 variant
  MISC_FEATURE (1)..(31): X is unnatural amino acid comprising tetrazine group or its variant, or triazine group or its variant.
HGEGTFTSDVSSXLEGQAAKEFIAWLVKGRX

SEQ ID NO: 15 - protein, 31 aa, Artificial Sequence
  GLP1 variant
  MISC_FEATURE (1)..(31): X is unnatural amino acid comprising tetrazine group or its variant, or triazine group or its variant.
HGEGTFTSDVSSYLEGQAAKEXIAWLVKGRX

SEQ ID NO: 16 - protein, 31 aa, Artificial Sequence
  GLP1 variant
  MISC_FEATURE (1)..(31): X is unnatural amino acid comprising tetrazine group or its variant, or triazine group or its variant.
HAEGTFTSDXSSXLEGQAAKEFIAWLVRGRG

SEQ ID NO: 17 - protein, 31 aa, Artificial Sequence
  GLP1 variant
  MISC_FEATURE (1)..(31): X is unnatural amino acid comprising tetrazine group or its variant, or triazine group or its variant.
HAEGTFTSDXSSYLEGQAAKEXIAWLVRGRG

SEQ ID NO: 18 - protein, 31 aa, Artificial Sequence
  GLP1 variant
  MISC_FEATURE (1)..(31): X is unnatural amino acid comprising tetrazine group or its variant, or triazine group or its variant.
HAEGTFTSDVSSXLEGQAAKEXIAWLVRGRG

SEQ ID NO: 19 - protein, 31 aa, Artificial Sequence
  GLP1 variant
  MISC_FEATURE (1)..(31): X is unnatural amino acid comprising tetrazine group or its variant, or triazine group or its variant.
HGEGTFTSDXSSXLEGQAAKEFIAWLVRGRG

SEQ ID NO: 20 - protein, 31 aa, Artificial Sequence
  GLP1 variant
  MISC_FEATURE (1)..(31): X is unnatural amino acid comprising tetrazine group or its variant, or triazine group or its variant.
HGEGTFTSDXSSXLEGQAAKEFIAWLVKGRX

SEQ ID NO: 21 - protein, 31 aa, Artificial Sequence
  GLP1 variant
  MISC_FEATURE (1)..(31): X is unnatural amino acid comprising tetrazine group or its variant, or triazine group or its variant.
HGEGTFTSDXSSYLEGQAAKEXIAWLVKGRX

SEQ ID NO: 22 - protein, 31 aa, Artificial Sequence
  GLP1 variant
  MISC_FEATURE (1)..(31): X is unnatural amino acid comprising tetrazine group or its variant, or triazine group or its variant.
HGEGTFTSDVSSXLEGQAAKEXIAWLVKGRX

SEQ ID NO: 23 - protein, 31 aa, Artificial Sequence
  GLP1 variant
  MISC_FEATURE (1)..(31): X is unnatural amino acid comprising tetrazine group or its variant, or triazine group or its variant.
HGEGTFTSDXSSYLEGQAAKEXIAWLVRGRG

SEQ ID NO: 24 - protein, 31 aa, Artificial Sequence
  GLP1 variant
  MISC_FEATURE (1)..(31): X is unnatural amino acid comprising tetrazine group or its variant, or triazine group or its variant.
HGEGTFTSDVSSXLEGQAAKEXIAWLVRGRG

SEQ ID NO: 25 - protein, 31 aa, Artificial Sequence
  GLP1 variant
  MISC_FEATURE (1)..(31): X is unnatural amino acid comprising tetrazine group or its variant, or triazine group or its variant.
HAEGTFTSDXSSXLEGQAAKEXIAWLVRGRG

SEQ ID NO: 26 - protein, 31 aa, Artificial Sequence; identical to SEQ ID NO: 2
  GLP1 variant
  MISC_FEATURE (1)..(31): X is unnatural amino acid comprising tetrazine group or its variant, or triazine group or its variant.

SEQ ID NO: 27 - protein, 191 aa, Artificial Sequence [sequence omitted]

SEQ ID NO: 28 - protein, 191 aa, Artificial Sequence
  hGH variant
  MISC_FEATURE (1)..(191): X is unnatural amino acid comprising tetrazine group or its variant, or triazine group or its variant.
FPTIPLSRLFDNAMLRAHRLHQLAFDTYXEFEEAYIPKEQKYSFLQNPQTSLCFSESIPTPSNREETQQKSNLELLRISLLLIQSWLEPVQFLRSVFANSLVYGASDSNVYDLLKDLEEGIQTLMGRLEDGSPRTGQIFKQTYSKFDTNSHNDDALLKNYGLLYCFRKDMDKVETFLRIVQCRSVEGSCGF

SEQ ID NO: 29 - protein, 191 aa, Artificial Sequence
  hGH variant
  MISC_FEATURE (1)..(191): X is unnatural amino acid comprising tetrazine group or its variant, or triazine group or its variant.
FPTIPLSRLFDNAMLRAHRLHQLAFDTYQEFEEAXIPKEQKYSFLQNPQTSLCFSESIPTPSNREETQQKSNLELLRISLLLIQSWLEPVQFLRSVFANSLVYGASDSNVYDLLKDLEEGIQTLMGRLEDGSPRTGQIFKQTYSKFDTNSHNDDALLKNYGLLYCFRKDMDKVETFLRIVQCRSVEGSCGF

SEQ ID NO: 30 - protein, 191 aa, Artificial Sequence
  hGH variant
  MISC_FEATURE (1)..(191): X is unnatural amino acid comprising tetrazine group or its variant, or triazine group or its variant.
FPTIPLSRLFDNAMLRAHRLHQLAFDTYQEFEEAYIPKEQKYSFLQNPQTSXCFSESIPTPSNREETQQKSNLELLRISLLLIQSWLEPVQFLRSVFANSLVYGASDSNVYDLLKDLEEGIQTLMGRLEDGSPRTGQIFKQTYSKFDTNSHNDDALLKNYGLLYCFRKDMDKVETFLRIVQCRSVEGSCGF

SEQ ID NO: 31 - protein, 191 aa, Artificial Sequence
  hGH variant
  MISC_FEATURE (1)..(191): X is unnatural amino acid comprising tetrazine group or its variant, or triazine group or its variant.
FPTIPLSRLFDNAMLRAHRLHQLAFDTYQEFEEAYIPKEQKYSFLQNPQTSLCFSXSIPTPSNREETQQKSNLELLRISLLLIQSWLEPVQFLRSVFANSLVYGASDSNVYDLLKDLEEGIQTLMGRLEDGSPRTGQIFKQTYSKFDTNSHNDDALLKNYGLLYCFRKDMDKVETFLRIVQCRSVEGSCGF

SEQ ID NO: 32 - protein, 191 aa, Artificial Sequence
  hGH variant
  MISC_FEATURE (1)..(191): X is unnatural amino acid comprising tetrazine group or its variant, or triazine group or its variant.
FPTIPLSRLFDNAMLRAHRLHQLAFDTYQEFEEAYIPKEQKYSFLQNPQTSLCFSESIPTPSNREXTQQKSNLELLRISLLLIQSWLEPVQFLRSVFANSLVYGASDSNVYDLLKDLEEGIQTLMGRLEDGSPRTGQIFKQTYSKFDTNSHNDDALLKNYGLLYCFRKDMDKVETFLRIVQCRSVEGSCGF

SEQ ID NO: 33 - protein, 191 aa, Artificial Sequence
  hGH variant
  MISC_FEATURE (1)..(191): X is unnatural amino acid comprising tetrazine group or its variant, or triazine group or its variant.
FPTIPLSRLFDNAMLRAHRLHQLAFDTYQEFEEAYIPKEQKYSFLQNPQTSLCFSESIPTPSNREETQXKSNLELLRISLLLIQSWLEPVQFLRSVFANSLVYGASDSNVYDLLKDLEEGIQTLMGRLEDGSPRTGQIFKQTYSKFDTNSHNDDALLKNYGLLYCFRKDMDKVETFLRIVQCRSVEGSCGF

SEQ ID NO: 34 - protein, 191 aa, Artificial Sequence
  hGH variant
  MISC_FEATURE (1)..(191): X is unnatural amino acid comprising tetrazine group or its variant, or triazine group or its variant.
FPTIPLSRLFDNAMLRAHRLHQLAFDTYQEFEEAYIPKEQKYSFLQNPQTSLCFSESIPTPSNREETQQKSNLXLLRISLLLIQSWLEPVQFLRSVFANSLVYGASDSNVYDLLKDLEEGIQTLMGRLEDGSPRTGQIFKQTYSKFDTNSHNDDALLKNYGLLYCFRKDMDKVETFLRIVQCRSVEGSCGF

SEQ ID NO: 35 - protein, 191 aa, Artificial Sequence
  hGH variant
  MISC_FEATURE (1)..(191): X is unnatural amino acid comprising tetrazine group or its variant, or triazine group or its variant.
FPTIPLSRLFDNAMLRAHRLHQLAFDTYQEFEEAYIPKEQKYSFLQNPQTSLCFSESIPTPSNREETQQKSNLELLRISLLLIQSWLEPVQXLRSVFANSLVYGASDSNVYDLLKDLEEGIQTLMGRLEDGSPRTGQIFKQTYSKFDTNSHNDDALLKNYGLLYCFRKDMDKVETFLRIVQCRSVEGSCGF

SEQ ID NO: 36 - protein, 191 aa, Artificial Sequence
  hGH variant
  MISC_FEATURE (1)..(191): X is unnatural amino acid comprising tetrazine group or its variant, or triazine group or its variant.
FPTIPLSRLFDNAMLRAHRLHQLAFDTYQEFEEAYIPKEQKYSFLQNPQTSLCFSESIPTPSNREETQQKSNLELLRISLLLIQSWLEPVQFLRSVFANSLVYGAXDSNVYDLLKDLEEGIQTLMGRLEDGSPRTGQIFKQTYSKFDTNSHNDDALLKNYGLLYCFRKDMDKVETFLRIVQCRSVEGSCGF

SEQ ID NO: 37 - protein, 191 aa, Artificial Sequence
  hGH variant
  MISC_FEATURE (1)..(191): X is unnatural amino acid comprising tetrazine group or its variant, or triazine group or its variant.
FPTIPLSRLFDNAMLRAHRLHQLAFDTYQEFEEAYIPKEQKYSFLQNPQTSLCFSESIPTPSNREETQQKSNLELLRISLLLIQSWLEPVQFLRSVFANSLVYGASDSNVYDLLKDLEEGIXTLMGRLEDGSPRTGQIFKQTYSKFDTNSHNDDALLKNYGLLYCFRKDMDKVETFLRIVQCRSVEGSCGF

SEQ ID NO: 38 - protein, 191 aa, Artificial Sequence
  hGH variant
  MISC_FEATURE (1)..(191): X is unnatural amino acid comprising tetrazine group or its variant, or triazine group or its variant.
FPTIPLSRLFDNAMLRAHRLHQLAFDTYQEFEEAYIPKEQKYSFLQNPQTSLCFSESIPTPSNREETQQKSNLELLRISLLLIQSWLEPVQFLRSVFANSLVYGASDSNVYDLLKDLEEGIQTLMGXLEDGSPRTGQIFKQTYSKFDTNSHNDDALLKNYGLLYCFRKDMDKVETFLRIVQCRSVEGSCGF

SEQ ID NO: 39 - protein, 191 aa, Artificial Sequence
  hGH variant
  MISC_FEATURE (1)..(191): X is unnatural amino acid comprising tetrazine group or its variant, or triazine group or its variant.
FPTIPLSRLFDNAMLRAHRLHQLAFDTYQEFEEAYIPKEQKYSFLQNPQTSLCFSESIPTPSNREETQQKSNLELLRISLLLIQSWLEPVQFLRSVFANSLVYGASDSNVYDLLKDLEEGIQTLMGRXEDGSPRTGQIFKQTYSKFDTNSHNDDALLKNYGLLYCFRKDMDKVETFLRIVQCRSVEGSCGF

SEQ ID NO: 40 - protein, 191 aa, Artificial Sequence
  hGH variant
  MISC_FEATURE (1)..(191): X is unnatural amino acid comprising tetrazine group or its variant, or triazine group or its variant.
FPTIPLSRLFDNAMLRAHRLHQLAFDTYQEFEEAYIPKEQKYSFLQNPQTSLCFSESIPTPSNREETQQKSNLELLRISLLLIQSWLEPVQFLRSVFANSLVYGASDSNVYDLLKDLEEGIQTLMGRLEDXSPRTGQIFKQTYSKFDTNSHNDDALLKNYGLLYCFRKDMDKVETFLRIVQCRSVEGSCGF

SEQ ID NO: 41 - protein, 191 aa, Artificial Sequence
  hGH variant
  MISC_FEATURE (1)..(191): X is unnatural amino acid comprising tetrazine group or its variant, or triazine group or its variant.
FPTIPLSRLFDNAMLRAHRLHQLAFDTYQEFEEAYIPKEQKYSFLQNPQTSLCFSESIPTPSNREETQQKSNLELLRISLLLIQSWLEPVQFLRSVFANSLVYGASDSNVYDLLKDLEEGIQTLMGRLEDGSPXTGQIFKQTYSKFDTNSHNDDALLKNYGLLYCFRKDMDKVETFLRIVQCRSVEGSCGF

SEQ ID NO: 42 - protein, 191 aa, Artificial Sequence
  hGH variant
  MISC_FEATURE (1)..(191): X is unnatural amino acid comprising tetrazine group or its variant, or triazine group or its variant.
FPTIPLSRLFDNAMLRAHRLHQLAFDTYQEFEEAYIPKEQKYSFLQNPQTSLCFSESIPTPSNREETQQKSNLELLRISLLLIQSWLEPVQFLRSVFANSLVYGASDSNVYDLLKDLEEGIQTLMGRLEDGSPRTGQIFKXTYSKFDTNSHNDDALLKNYGLLYCFRKDMDKVETFLRIVQCRSVEGSCGF

SEQ ID NO: 43 - protein, 191 aa, Artificial Sequence
  hGH variant
  MISC_FEATURE (1)..(191): X is unnatural amino acid comprising tetrazine group or its variant, or triazine group or its variant.
FPTIPLSRLFDNAMLRAHRLHQLAFDTYQEFEEAYIPKEQKYSFLQNPQTSLCFSESIPTPSNREETQQKSNLELLRISLLLIQSWLEPVQFLRSVFANSLVYGASDSNVYDLLKDLEEGIQTLMGRLEDGSPRTGQIFKQXYSKFDTNSHNDDALLKNYGLLYCFRKDMDKVETFLRIVQCRSVEGSCGF

SEQ ID NO: 44 - protein, 191 aa, Artificial Sequence
  hGH variant
  MISC_FEATURE (1)..(191): X is unnatural amino acid comprising tetrazine group or its variant, or triazine group or its variant.
FPTIPLSRLFDNAMLRAHRLHQLAFDTYQEFEEAYIPKEQKYSFLQNPQTSLCFSESIPTPSNREETQQKSNLELLRISLLLIQSWLEPVQFLRSVFANSLVYGASDSNVYDLLKDLEEGIQTLMGRLEDGSPRTGQIFKQTXSKFDTNSHNDDALLKNYGLLYCFRKDMDKVETFLRIVQCRSVEGSCGF

SEQ ID NO: 45 - protein, 191 aa, Artificial Sequence
  hGH variant
  MISC_FEATURE (1)..(191): X is unnatural amino acid comprising tetrazine group or its variant, or triazine group or its variant.
FPTIPLSRLFDNAMLRAHRLHQLAFDTYQEFEEAYIPKEQKYSFLQNPQTSLCFSESIPTPSNREETQQKSNLELLRISLLLIQSWLEPVQFLRSVFANSLVYGASDSNVYDLLKDLEEGIQTLMGRLEDGSPRTGQIFKQTYSXFDTNSHNDDALLKNYGLLYCFRKDMDKVETFLRIVQCRSVEGSCGF

SEQ ID NO: 46 - protein, 191 aa, Artificial Sequence
  hGH variant
  MISC_FEATURE (1)..(191): X is unnatural amino acid comprising tetrazine group or its variant, or triazine group or its variant.
FPTIPLSRLFDNAMLRAHRLHQLAFDTYQEFEEAYIPKEQKYSFLQNPQTSLCFSESIPTPSNREETQQKSNLELLRISLLLIQSWLEPVQFLRSVFANSLVYGASDSNVYDLLKDLEEGIQTLMGRLEDGSPRTGQIFKQTYSKFXTNSHNDDALLKNYGLLYCFRKDMDKVETFLRIVQCRSVEGSCGF

SEQ ID NO: 47 - protein, 191 aa, Artificial Sequence
  hGH variant
  MISC_FEATURE (1)..(191): X is unnatural amino acid comprising tetrazine group or its variant, or triazine group or its variant.
FPTIPLSRLFDNAMLRAHRLHQLAFDTYQEFEEAYIPKEQKYSFLQNPQTSLCFSESIPTPSNREETQQKSNLELLRISLLLIQSWLEPVQFLRSVFANSLVYGASDSNVYDLLKDLEEGIQTLMGRLEDGSPRTGQIFKQTYSKFDTXSHNDDALLKNYGLLYCFRKDMDKVETFLRIVQCRSVEGSCGF

SEQ ID NO: 48 - protein, 191 aa, Artificial Sequence
  hGH variant
  MISC_FEATURE (1)..(191): X is unnatural amino acid comprising tetrazine group or its variant, or triazine group or its variant.
FPTIPLSRLFDNAMLRAHRLHQLAFDTYQEFEEAYIPKEQKYSFLQNPQTSLCFSESIPTPSNREETQQKSNLELLRISLLLIQSWLEPVQFLRSVFANSLVYGASDSNVYDLLKDLEEGIQTLMGRLEDGSPRTGQIFKQTYSKFDTNSHXDDALLKNYGLLYCFRKDMDKVETFLRIVQCRSVEGSCGF

SEQ ID NO: 49 - protein, 191 aa, Artificial Sequence
  hGH variant
  MISC_FEATURE (1)..(191): X is unnatural amino acid comprising tetrazine group or its variant, or triazine group or its variant.
FPTIPLSRLFDNAMLRAHRLHQLAFDTYQEFEEAYIPKEQKYSFLQNPQTSLCFSESIPTPSNREETQQKSNLELLRISLLLIQSWLEPVQFLRSVFANSLVYGASDSNVYDLLKDLEEGIQTLMGRLEDGSPRTGQIFKQTYSKFDTNSHNXDALLKNYGLLYCFRKDMDKVETFLRIVQCRSVEGSCGF

SEQ ID NO: 50 - protein, 191 aa, Artificial Sequence
  hGH variant
  MISC_FEATURE (1)..(191): X is unnatural amino acid comprising tetrazine group or its variant, or triazine group or its variant.
FPTIPLSRLFDNAMLRAHRLHQLAFDTYQEFEEAYIPKEQKYSFLQNPQTSLCFSESIPTPSNREETQQKSNLELLRISLLLIQSWLEPVQFLRSVFANSLVYGASDSNVYDLLKDLEEGIQTLMGRLEDGSPRTGQIFKQTYSKFDTNSHNDDALLKNYGLLYCFRKDMDKVETFLRIVQCRSVXGSCGF

SEQ ID NO: 51 - protein, 238 aa, Artificial Sequence
  sfGFP
GSMSKGEELFTGVVPILVELDGDVNGHKFSVRGEGEGDATNGKLTLKFICTTGKLPVPWPTLVTTLTYGVQCFSRYPDHMKRHDFFKSAMPEGYVQERTISFKDDGTYKTRAEVKFEGDTLVNRIELKGIDFKEDGNILGHKLEYNFNSHNVYITADKQKNGIKANFKIRHNVEDGSVQLADHYQQNTPIGDGPVLLPDNHYLSTQSVLSKDPNEKRDHMVLLEFVTAAGITHGMDEL

SEQ ID NO: 52 - protein, 238 aa, Artificial Sequence
  sfGFP variant
  MISC_FEATURE (1)..(238): X is unnatural amino acid comprising tetrazine group or its variant, or triazine group or its variant.
GSMSKGEXLFTGVVPILVELDGDVNGHKFSVRGEGEGDATNGKLTLKFICTTGKLPVPWPTLVTTLTYGVQCFSRYPDHMKRHDFFKSAMPEGYVQERTISFKDDGTYKTRAEVKFEGDTLVNRIELKGIDFKEDGNILGHKLEYNFNSHNVYITADKQKNGIKANFKIRHNVEDGSVQLADHYQQNTPIGDGPVLLPDNHYLSTQSVLSKDPNEKRDHMVLLEFVTAAGITHGMDEL

SEQ ID NO: 53 - protein, 238 aa, Artificial Sequence
  sfGFP variant
  MISC_FEATURE (1)..(238): X is unnatural amino acid comprising tetrazine group or its variant, or triazine group or its variant.
GSMSKGEELFXGVVPILVELDGDVNGHKFSVRGEGEGDATNGKLTLKFICTTGKLPVPWPTLVTTLTYGVQCFSRYPDHMKRHDFFKSAMPEGYVQERTISFKDDGTYKTRAEVKFEGDTLVNRIELKGIDFKEDGNILGHKLEYNFNSHNVYITADKQKNGIKANFKIRHNVEDGSVQLADHYQQNTPIGDGPVLLPDNHYLSTQSVLSKDPNEKRDHMVLLEFVTAAGITHGMDEL

SEQ ID NO: 54 - protein, 238 aa, Artificial Sequence
  sfGFP variant
  MISC_FEATURE (1)..(238): X is unnatural amino acid comprising tetrazine group or its variant, or triazine group or its variant.
GSMSKGEELFTGXVPILVELDGDVNGHKFSVRGEGEGDATNGKLTLKFICTTGKLPVPWPTLVTTLTYGVQCFSRYPDHMKRHDFFKSAMPEGYVQERTISFKDDGTYKTRAEVKFEGDTLVNRIELKGIDFKEDGNILGHKLEYNFNSHNVYITADKQKNGIKANFKIRHNVEDGSVQLADHYQQNTPIGDGPVLLPDNHYLSTQSVLSKDPNEKRDHMVLLEFVTAAGITHGMDEL

SEQ ID NO: 55 - protein, 238 aa, Artificial Sequence
  sfGFP variant
  MISC_FEATURE (1)..(238): X is unnatural amino acid comprising tetrazine group or its variant, or triazine group or its variant.
GSMSKGEELFTGVVPILVELDGDVNXHKFSVRGEGEGDATNGKLTLKFICTTGKLPVPWPTLVTTLTYGVQCFSRYPDHMKRHDFFKSAMPEGYVQERTISFKDDGTYKTRAEVKFEGDTLVNRIELKGIDFKEDGNILGHKLEYNFNSHNVYITADKQKNGIKANFKIRHNVEDGSVQLADHYQQNTPIGDGPVLLPDNHYLSTQSVLSKDPNEKRDHMVLLEFVTAAGITHGMDEL

SEQ ID NO: 56 - protein, 238 aa, Artificial Sequence
  sfGFP variant
  MISC_FEATURE (1)..(238): X is unnatural amino acid comprising tetrazine group or its variant, or triazine group or its variant.
GSMSKGEELFTGVVPILVELDGDVNGHXFSVRGEGEGDATNGKLTLKFICTTGKLPVPWPTLVTTLTYGVQCFSRYPDHMKRHDFFKSAMPEGYVQERTISFKDDGTYKTRAEVKFEGDTLVNRIELKGIDFKEDGNILGHKLEYNFNSHNVYITADKQKNGIKANFKIRHNVEDGSVQLADHYQQNTPIGDGPVLLPDNHYLSTQSVLSKDPNEKRDHMVLLEFVTAAGITHGMDEL

SEQ ID NO: 57 - protein, 238 aa, Artificial Sequence
  sfGFP variant
  MISC_FEATURE (1)..(238): X is unnatural amino acid comprising tetrazine group or its variant, or triazine group or its variant.
GSMSKGEELFTGVVPILVELDGDVNGHKFSVRGEGEGDAXNGKLTLKFICTTGKLPVPWPTLVTTLTYGVQCFSRYPDHMKRHDFFKSAMPEGYVQERTISFKDDGTYKTRAEVKFEGDTLVNRIELKGIDFKEDGNILGHKLEYNFNSHNVYITADKQKNGIKANFKIRHNVEDGSVQLADHYQQNTPIGDGPVLLPDNHYLSTQSVLSKDPNEKRDHMVLLEFVTAAGITHGMDEL

SEQ ID NO: 58 - protein, 238 aa, Artificial Sequence
  sfGFP variant
  MISC_FEATURE (1)..(238): X is unnatural amino acid comprising tetrazine group or its variant, or triazine group or its variant.
GSMSKGEELFTGVVPILVELDGDVNGHKFSVRGEGEGDATXGKLTLKFICTTGKLPVPWPTLVTTLTYGVQCFSRYPDHMKRHDFFKSAMPEGYVQERTISFKDDGTYKTRAEVKFEGDTLVNRIELKGIDFKEDGNILGHKLEYNFNSHNVYITADKQKNGIKANFKIRHNVEDGSVQLADHYQQNTPIGDGPVLLPDNHYLSTQSVLSKDPNEKRDHMVLLEFVTAAGITHGMDEL

SEQ ID NO: 59 - protein, 238 aa, Artificial Sequence
  sfGFP variant
  MISC_FEATURE (1)..(238): X is unnatural amino acid comprising tetrazine group or its variant, or triazine group or its variant.
GSMSKGEELFTGVVPILVELDGDVNGHKFSVRGEGEGDATNGKLTLKFICXTGKLPVPWPTLVTTLTYGVQCFSRYPDHMKRHDFFKSAMPEGYVQERTISFKDDGTYKTRAEVKFEGDTLVNRIELKGIDFKEDGNILGHKLEYNFNSHNVYITADKQKNGIKANFKIRHNVEDGSVQLADHYQQNTPIGDGPVLLPDNHYLSTQSVLSKDPNEKRDHMVLLEFVTAAGITHGMDEL

SEQ ID NO: 60 - protein, 238 aa, Artificial Sequence
  sfGFP variant
  MISC_FEATURE (1)..(238): X is unnatural amino acid comprising tetrazine group or its variant, or triazine group or its variant.
GSMSKGEELFTGVVPILVELDGDVNGHKFSVRGEGEGDATNGKLTLKFICTTGKLPVPWPTLVTTLTYGVQCFSRYPXHMKRHDFFKSAMPEGYVQERTISFKDDGTYKTRAEVKFEGDTLVNRIELKGIDFKEDGNILGHKLEYNFNSHNVYITADKQKNGIKANFKIRHNVEDGSVQLADHYQQNTPIGDGPVLLPDNHYLSTQSVLSKDPNEKRDHMVLLEFVTAAGITHGMDEL

SEQ ID NO: 61 - protein, 238 aa, Artificial Sequence
  sfGFP variant
  MISC_FEATURE (1)..(238): X is unnatural amino acid comprising tetrazine group or its variant, or triazine group or its variant.
GSMSKGEELFTGVVPILVELDGDVNGHKFSVRGEGEGDATNGKLTLKFICTTGKLPVPWPTLVTTLTYGVQCFSRYPDHMKRHDFFKSAMPEGYVQERTISFXDDGTYKTRAEVKFEGDTLVNRIELKGIDFKEDGNILGHKLEYNFNSHNVYITADKQKNGIKANFKIRHNVEDGSVQLADHYQQNTPIGDGPVLLPDNHYLSTQSVLSKDPNEKRDHMVLLEFVTAAGITHGMDEL

SEQ ID NO: 62 - protein, 238 aa, Artificial Sequence
  sfGFP variant
  MISC_FEATURE (1)..(238): X is unnatural amino acid comprising tetrazine group or its variant, or triazine group or its variant.
GSMSKGEELFTGVVPILVELDGDVNGHKFSVRGEGEGDATNGKLTLKFICTTGKLPVPWPTLVTTLTYGVQCFSRYPDHMKRHDFFKSAMPEGYVQERTISFKDDGTYXTRAEVKFEGDTLVNRIELKGIDFKEDGNILGHKLEYNFNSHNVYITADKQKNGIKANFKIRHNVEDGSVQLADHYQQNTPIGDGPVLLPDNHYLSTQSVLSKDPNEKRDHMVLLEFVTAAGITHGMDEL

SEQ ID NO: 63 - protein, 238 aa, Artificial Sequence
  sfGFP variant
  MISC_FEATURE (1)..(238): X is unnatural amino acid comprising tetrazine group or its variant, or triazine group or its variant.
GSMSKGEELFTGVVPILVELDGDVNGHKFSVRGEGEGDATNGKLTLKFICTTGKLPVPWPTLVTTLTYGVQCFSRYPDHMKRHDFFKSAMPEGYVQERTISFKDDGTYKTRAEVKFEXDTLVNRIELKGIDFKEDGNILGHKLEYNFNSHNVYITADKQKNGIKANFKIRHNVEDGSVQLADHYQQNTPIGDGPVLLPDNHYLSTQSVLSKDPNEKRDHMVLLEFVTAAGITHGMDEL

SEQ ID NO: 64 - protein, 238 aa, Artificial Sequence
  sfGFP variant
  MISC_FEATURE (1)..(238): X is unnatural amino acid comprising tetrazine group or its variant, or triazine group or its variant.
GSMSKGEELFTGVVPILVELDGDVNGHKFSVRGEGEGDATNGKLTLKFICTTGKLPVPWPTLVTTLTYGVQCFSRYPDHMKRHDFFKSAMPEGYVQERTISFKDDGTYKTRAEVKFEGDTLVNRIELXGIDFKEDGNILGHKLEYNFNSHNVYITADKQKNGIKANFKIRHNVEDGSVQLADHYQQNTPIGDGPVLLPDNHYLSTQSVLSKDPNEKRDHMVLLEFVTAAGITHGMDEL

SEQ ID NO: 65 - protein, 238 aa, Artificial Sequence
  sfGFP variant
  MISC_FEATURE (1)..(238): X is unnatural amino acid comprising tetrazine group or its variant, or triazine group or its variant.
GSMSKGEELFTGVVPILVELDGDVNGHKFSVRGEGEGDATNGKLTLKFICTTGKLPVPWPTLVTTLTYGVQCFSRYPDHMKRHDFFKSAMPEGYVQERTISFKDDGTYKTRAEVKFEGDTLVNRIELKGIXFKEDGNILGHKLEYNFNSHNVYITADKQKNGIKANFKIRHNVEDGSVQLADHYQQNTPIGDGPVLLPDNHYLSTQSVLSKDPNEKRDHMVLLEFVTAAGITHGMDEL

SEQ ID NO: 66 - protein, 238 aa, Artificial Sequence
  sfGFP variant
  MISC_FEATURE (1)..(238): X is unnatural amino acid comprising tetrazine group or its variant, or triazine group or its variant.
GSMSKGEELFTGVVPILVELDGDVNGHKFSVRGEGEGDATNGKLTLKFICTTGKLPVPWPTLVTTLTYGVQCFSRYPDHMKRHDFFKSAMPEGYVQERTISFKDDGTYKTRAEVKFEGDTLVNRIELKGIDFKEXGNILGHKLEYNFNSHNVYITADKQKNGIKANFKIRHNVEDGSVQLADHYQQNTPIGDGPVLLPDNHYLSTQSVLSKDPNEKRDHMVLLEFVTAAGITHGMDEL

SEQ ID NO: 67 - protein, 238 aa, Artificial Sequence
  sfGFP variant
  MISC_FEATURE (1)..(238): X is unnatural amino acid comprising tetrazine group or its variant, or triazine group or its variant.
GSMSKGEELFTGVVPILVELDGDVNGHKFSVRGEGEGDATNGKLTLKFICTTGKLPVPWPTLVTTLTYGVQCFSRYPDHMKRHDFFKSAMPEGYVQERTISFKDDGTYKTRAEVKFEGDTLVNRIELKGIDFKEDGNILGHKLEYNFNSXNVYITADKQKNGIKANFKIRHNVEDGSVQLADHYQQNTPIGDGPVLLPDNHYLSTQSVLSKDPNEKRDHMVLLEFVTAAGITHGMDEL

SEQ ID NO: 68 - protein, 238 aa, Artificial Sequence
  sfGFP variant
  MISC_FEATURE (1)..(238): X is unnatural amino acid comprising tetrazine group or its variant, or triazine group or its variant.
GSMSKGEELFTGVVPILVELDGDVNGHKFSVRGEGEGDATNGKLTLKFICTTGKLPVPWPTLVTTLTYGVQCFSRYPDHMKRHDFFKSAMPEGYVQERTISFKDDGTYKTRAEVKFEGDTLVNRIELKGIDFKEDGNILGHKLEYNFNSHNVYITADKXKNGIKANFKIRHNVEDGSVQLADHYQQNTPIGDGPVLLPDNHYLSTQSVLSKDPNEKRDHMVLLEFVTAAGITHGMDEL

SEQ ID NO: 69 - protein, 238 aa, Artificial Sequence
  sfGFP variant
  MISC_FEATURE (1)..(238): X is unnatural amino acid comprising tetrazine group or its variant, or triazine group or its variant.
GSMSKGEELFTGVVPILVELDGDVNGHKFSVRGEGEGDATNGKLTLKFICTTGKLPVPWPTLVTTLTYGVQCFSRYPDHMKRHDFFKSAMPEGYVQERTISFKDDGTYKTRAEVKFEGDTLVNRIELKGIDFKEDGNILGHKLEYNFNSHNVYITADKQKNGIKANFXIRHNVEDGSVQLADHYQQNTPIGDGPVLLPDNHYLSTQSVLSKDPNEKRDHMVLLEFVTAAGITHGMDEL

SEQ ID NO: 70 - protein, 238 aa, Artificial Sequence
  sfGFP variant
  MISC_FEATURE (1)..(238): X is unnatural amino acid comprising tetrazine group or its variant, or triazine group or its variant.
GSMSKGEELFTGVVPILVELDGDVNGHKFSVRGEGEGDATNGKLTLKFICTTGKLPVPWPTLVTTLTYGVQCFSRYPDHMKRHDFFKSAMPEGYVQERTISFKDDGTYKTRAEVKFEGDTLVNRIELKGIDFKEDGNILGHKLEYNFNSHNVYITADKQKNGIKANFKIRHNVEXGSVQLADHYQQNTPIGDGPVLLPDNHYLSTQSVLSKDPNEKRDHMVLLEFVTAAGITHGMDEL

SEQ ID NO: 71 - protein, 238 aa, Artificial Sequence
  sfGFP variant
  MISC_FEATURE (1)..(238): X is unnatural amino acid comprising tetrazine group or its variant, or triazine group or its variant.
GSMSKGEELFTGVVPILVELDGDVNGHKFSVRGEGEGDATNGKLTLKFICTTGKLPVPWPTLVTTLTYGVQCFSRYPDHMKRHDFFKSAMPEGYVQERTISFKDDGTYKTRAEVKFEGDTLVNRIELKGIDFKEDGNILGHKLEYNFNSHNVYITADKQKNGIKANFKIRHNVEDGSVQLADHYQQNTPIGXGPVLLPDNHYLSTQSVLSKDPNEKRDHMVLLEFVTAAGITHGMDEL

SEQ ID NO: 72 - protein, 238 aa, Artificial Sequence
  sfGFP variant
  MISC_FEATURE (1)..(238): X is unnatural amino acid comprising tetrazine group or its variant, or triazine group or its variant.
GSMSKGEELFTGVVPILVELDGDVNGHKFSVRGEGEGDATNGKLTLKFICTTGKLPVPWPTLVTTLTYGVQCFSRYPDHMKRHDFFKSAMPEGYVQERTISFKDDGTYKTRAEVKFEGDTLVNRIELKGIDFKEDGNILGHKLEYNFNSHNVYITADKQKNGIKANFKIRHNVEDGSVQLADHYQQNTPIGDGPXLLPDNHYLSTQSVLSKDPNEKRDHMVLLEFVTAAGITHGMDEL

SEQ ID NO: 73 - protein, 238 aa, Artificial Sequence
  sfGFP variant
  MISC_FEATURE (1)..(238): X is unnatural amino acid comprising tetrazine group or its variant, or triazine group or its variant.
GSMSKGEELFTGVVPILVELDGDVNGHKFSVRGEGEGDATNGKLTLKFICTTGKLPVPWPTLVTTLTYGVQCFSRYPDHMKRHDFFKSAMPEGYVQERTISFKDDGTYKTRAEVKFEGDTLVNRIELKGIDFKEDGNILGHKLEYNFNSHNVYITADKQKNGIKANFKIRHNVEDGSVQLADHYQQNTPIGDGPVLLPDXHYLSTQSVLSKDPNEKRDHMVLLEFVTAAGITHGMDEL

SEQ ID NO: 74 - protein, 238 aa, Artificial Sequence
  sfGFP variant
  MISC_FEATURE (1)..(238): X is unnatural amino acid comprising tetrazine group or its variant, or triazine group or its variant.
GSMSKGEELFTGVVPILVELDGDVNGHKFSVRGEGEGDATNGKLTLKFICTTGKLPVPWPTLVTTLTYGVQCFSRYPDHMKRHDFFKSAMPEGYVQERTISFKDDGTYKTRAEVKFEGDTLVNRIELKGIDFKEDGNILGHKLEYNFNSHNVYITADKQKNGIKANFKIRHNVEDGSVQLADHYQQNTPIGDGPVLLPDNHYLSTQSVLSKDXNEKRDHMVLLEFVTAAGITHGMDEL

SEQ ID NO: 75 - protein, 238 aa, Artificial Sequence
  sfGFP variant
  MISC_FEATURE (1)..(238): X is unnatural amino acid comprising tetrazine group or its variant, or triazine group or its variant.
GSMSKGEELFTGVVPILVELDGDVNGHKFSVRGEGEGDATNGKLTLKFICTTGKLPVPWPTLVTTLTYGVQCFSRYPDHMKRHDFFKSAMPEGYVQERTISFKDDGTYKTRAEVKFEGDTLVNRIELKGIDFKEDGNILGHKLEYNFNSHNVYITADKQKNGIKANFKIRHNVEDGSVQLADHYQQNTPIGDGPVLLPDNHYLSTQSVLSKDPNEKRDHMVLLEFVTAAXITHGMDEL

SEQ ID NO: 76 - protein, 585 aa, Artificial Sequence [sequence omitted]

SEQ ID NO: 77 - protein, 585 aa, Artificial Sequence
  HSA variant
DAHKSEVAHRFKDLGEENFKALVLIAFAQYLQQCPFEDHVKLVNEVTEFAKTCVADESAENCDKSLHTLFGDKLCTVATLRETYGEMADCCAKQEPERNECFLQHKDDNPNLPRLVRPEVDVMCTAFHDNEETFLKKYLYEIARRHPYFYAPELLFFAKRYKAAFTECCQAADKAACLLPKLDELRDEGKASSAKQRLKCASLQKFGERAFKAWAVARLSQRFPKAEFAEVSKLVTDLTKVHTECCHGDLLECADDRADLAKYICENQDSISSKLKECCEKPLLEKSHCIAEVENDEMPADLPSLAADFVESKDVCKNYAEAKDVFLGMFLYEYARRHPDYSVVLLLRLAKTYETTLEKCCAAADPHECYAKVFDEFKPLVEEPQNLIKQNCELFEQLGEYKFQNALLVRYTKKVPQMSTPTLVEVSRNLGKVGSKCCKHPEAKRMPCAEDYLSVVLNQLCVLHEKTPVSDRVTKCCTESLVNRRPCFSALEVDETYVPKEFNAETFTFHADICTLSEKERQIKKQTALVELVKHKPKATKEQLKAVMDDFAAFVEKCCKADDKETCFAEEGKKLVAASQAALGL

SEQ ID NO: 78 - protein, 585 aa, Artificial Sequence
  HSA variant
DAHKSEVAHRFKDLGEENFKALVLIAFAQYLQQCPFEDHVKLVNEVTEFAKTCVADESAENCDKSLHTLFGDKLCTVATLRETYGEMADCCAKQEPERNECFLQHKDDNPNLPRLVRPEVDVMCTAFHDNEETFLKKYLYEIARRHPYFYAPELLFFAKRYKAAFTECCQAADKAACLLPKLDELRDEGKASSAKQRLKCASLQKFGERAFKAWAVARLSQRFPKAEFAEVSKLVTDLTKVHTECCHGDLLECADDRADLAKYICENQDSISSKLKECCEKPLLEKSHCIAEVENDEMPADLPSLAADFVESKDVCKNYAEAKDVFLGMFLYEYARRHPDYSVVLLLRLAKTYETTLEKCCAAADPHECYAKVFDEFKPLVEEPQNLIKQNCELFEQLGEYKFQNALLVRYTKKVPQVSAPTLVEVSRNLGKVGSKCCKHPEAKRMPCAEDYLSVVLNQLCVLHEKTPVSDRVTKCCTESLVNRRPCFSALEVDETYVPKEFNAETFTFHADICTLSEKERQIKKQTALVELVKHKPKATKEQLKAVMDDFAAFVEKCCKADDKETCFAEEGKKLVAASQAALGL

SEQ ID NO: 79 - protein, 585 aa, Artificial Sequence
  HSA variant
DAHKSEVAHRFKDLGEENFKALVLIAFAQYLQQCPFEDHVKLVNEVTEFAKTCVADESAENCDKSLHTLFGDKLCTVATLRETYGEMADCCAKQEPERNECFLQHKDDNPNLPRLVRPEVDVMCTAFHDNEETFLKKYLYEIARRHPYFYAPELLFFAKRYKAAFTECCQAADKAACLLPKLDELRDEGKASSAKQRLKCASLQKFGERAFKAWAVARLSQRFPKAEFAEVSKLVTDLTKVHTECCHGDLLECADDRADLAKYICENQDSISSKLKECCEKPLLEKSHCIAEVENDEMPADLPSLAADFVESKDVCKNYAEAKDVFLGMFLYEYARRHPDYSVVLLLRLAKTYETTLEKCCAAADPHECYAKVFDEFKPLVEEPQNLIKQNCELFEQLGEYKFQNALLVRYTKKVPQVSTPTLVEVSRNLGKVGSKCCKHPEAKRMPCAEDYLSVVLNQLCVLHEKTPVSDRVTKCCTESLVNRRPCFSALEVDETYVPKEFNARTFTFHADICTLSEKERQIKKQTALVELVKHKPKATKEQLKAVMDDFAAFVEKCCKADDKETCFAEEGKKLVAASQAALGL

SEQ ID NO: 80 - protein, 585 aa, Artificial Sequence
  HSA variant
DAHKSEVAHRFKDLGEENFKALVLIAFAQYLQQCPFEDHVKLVNEVTEFAKTCVADESAENCDKSLHTLFGDKLCTVATLRETYGEMADCCAKQEPERNECFLQHKDDNPNLPRLVRPEVDVMCTAFHDNEETFLKKYLYEIARRHPYFYAPELLFFAKRYKAAFTECCQAADKAACLLPKLDELRDEGKASSAKQRLKCASLQKFGERAFKAWAVARLSQRFPKAEFAEVSKLVTDLTKVHTECCHGDLLECADDRADLAKYICENQDSISSKLKECCEKPLLEKSHCIAEVENDEMPADLPSLAADFVESKDVCKNYAEAKDVFLGMFLYEYARRHPDYSVVLLLRLAKTYETTLEKCCAAADPHECYAKVFDEFKPLVEEPQNLIKQNCELFEQLGEYKFQNALLVRYTKKVPQVSTPTLVEVSRNLGKVGSKCCKHPEAKRMPCAEDYLSVVLNQLCVLHEKTPVSDRVTKCCTESLVNRRPCFSALEVDETYVPKEFNAGTFTFHADICTLSEKERQIKKQTALVELVKHKPKATKEQLKAVMDDFAAFVEKCCKADDKETCFAEEGKKLVAASQAALGL

SEQ ID NO: 81 - protein, 585 aa, Artificial Sequence
  HSA variant
DAHKSEVAHRFKDLGEENFKALVLIAFAQYLQQCPFEDHVKLVNEVTEFAKTCVADESAENCDKSLHTLFGDKLCTVATLRETYGEMADCCAKQEPERNECFLQHKDDNPNLPRLVRPEVDVMCTAFHDNEETFLKKYLYEIARRHPYFYAPELLFFAKRYKAAFTECCQAADKAACLLPKLDELRDEGKASSAKQRLKCASLQKFGERAFKAWAVARLSQRFPKAEFAEVSKLVTDLTKVHTECCHGDLLECADDRADLAKYICENQDSISSKLKECCEKPLLEKSHCIAEVENDEMPADLPSLAADFVESKDVCKNYAEAKDVFLGMFLYEYARRHPDYSVVLLLRLAKTYETTLEKCCAAADPHECYAKVFDEFKPLVEEPQNLIKQNCELFEQLGEYKFQNALLVRYTKKVPQVSTPTLVEVSRNLGKVGSKCCKHPEAKRMPCAEDYLSVVLNQLCVLHEKTPVSDRVTKCCTESLVNRRPCFSALEVDETYVPKEFNAETFTFHADICTLSEKERQIKKQTALVELVKHKPKATKEQLKAAMDDFAAFVEKCCKADDKETCFAEEGKKLVAASQAALGL

SEQ ID NO: 82 - protein, 585 aa, Artificial Sequence
  HSA variant
DAHKSEVAHRFKDLGEENFKALVLIAFAQYLQQCPFEDHVKLVNEVTEFAKTCVADESAENCDKSLHTLFGDKLCTVATLRETYGEMADCCAKQEPERNECFLQHKDDNPNLPRLVRPEVDVMCTAFHDNEETFLKKYLYEIARRHPYFYAPELLFFAKRYKAAFTECCQAADKAACLLPKLDELRDEGKASSAKQRLKCASLQKFGERAFKAWAVARLSQRFPKAEFAEVSKLVTDLTKVHTECCHGDLLECADDRADLAKYICENQDSISSKLKECCEKPLLEKSHCIAEVENDEMPADLPSLAADFVESKDVCKNYAEAKDVFLGMFLYEYARRHPDYSVVLLLRLAKTYETTLEKCCAAADPHECYAKVFDEFKPLVEEPQNLIKQNCELFEQLGEYKFQNALLVRYTKKVPQVSTPTLVEVSRNLGKVGSKCCKHPEAKRMPCAEDYLSVVLNQLCVLHEKTPVSDRVTKCCTESLVNRRPCFSALEVDETYVPKEFNAETFTFHADICTLSEKERQIKKQTALVELVKHKPKATKEQLKAVMDDFAAFVEKCCKADDKETCFAEEGYKLVAASQAALGL

SEQ ID NO: 83 - protein, 585 aa, Artificial Sequence
  HSA variant
DAHKSEVAHRFKDLGEENFKALVLIAFAQYLQQCPFEDHVKLVNEVTEFAKTCVADESAENCDKSLHTLFGDKLCTVATLRETYGEMADCCAKQEPERNECFLQHKDDNPNLPRLVRPEVDVMCTAFHDNEETFLKKYLYEIARRHPYFYAPELLFFAKRYKAAFTECCQAADKAACLLPKLDELRDEGKASSAKQRLKCASLQKFGERAFKAWAVARLSQRFPKAEFAEVSKLVTDLTKVHTECCHGDLLECADDRADLAKYICENQDSISSKLKECCEKPLLEKSHCIAEVENDEMPADLPSLAADFVESKDVCKNYAEAKDVFLGMFLYEYARRHPDYSVVLLLRLAKTYETTLEKCCAAADPHECYAKVFDEFKPLVEEPQNLIKQNCELFEQLGEYKFQNALLVRYTKKVPQVSTPTLIEVSRNLGKVGSKCCKHPEAKRMPCAEDYLSVVLNQLCVLHEKTPVSDRVTKCCTESLVNRRPCFSALEVDETYVPKEFNAETFTFHADICTLSEKERQIKKQTALVELVKHKPKATKEQLKAVMDDFAAFVEKCCKADDKETCFAEEGKKLVAASQAALGL

SEQ ID NO: 84 - protein, 585 aa, Artificial Sequence
  HSA variant
DAHKSEVAHRFKDLGEENFKALVLIAFAQYLQQCPFEDHVKLVNEVTEFAKTCVADESAENCDKSLHTLFGDKLCTVATLRETYGEMADCCAKQEPERNECFLQHKDDNPNLPRLVRPEVDVMCTAFHDNEETFLKKYLYEIARRHPYFYAPELLFFAKRYKAAFTECCQAADKAACLLPKLDELRDEGKASSAKQRLKCASLQKFGERAFKAWAVARLSQRFPKAEFAEVSKLVTDLTKVHTECCHGDLLECADDRADLAKYICENQDSISSKLKECCEKPLLEKSHCIAEVENDEMPADLPSLAADFVESKDVCKNYAEAKDVFLGMFLYEYARRHPDYSVVLLLRLAKTYETTLEKCCAAADPHECYAKVFDEFKPLVEEPQNLIKQNCELFEQLGEYKFQNALLVRYTKKVPQVSTPTLVEVSRDLGKVGSKCCKHPEAKRMPCAEDYLSVVLNQLCVLHEKTPVSDRVTKCCTESLVNRRPCFSALEVDETYVPKEFNAETFTFHADICTLSEKERQIKKQTALVELVKHKPKATKEQLKAVMDDFAAFVEKCCKADDKETCFAEEGKKLVAASQAALGL

SEQ ID NO: 85 - protein, 585 aa, Artificial Sequence
  HSA variant
DAHKSEVAHRFKDLGEENFKALVLIAFAQYLQQCPFEDHVKLVNEVTEFAKTCVADESAENCDKSLHTLFGDKLCTVATLRETYGEMADCCAKQEPERNECFLQHKDDNPNLPRLVRPEVDVMCTAFHDNEETFLKKYLYEIARRHPYFYAPELLFFAKRYKAAFTECCQAADKAACLLPKLDELRDEGKASSAKQRLKCASLQKFGERAFKAWAVARLSQRFPKAEFAEVSKLVTDLTKVHTECCHGDLLECADDRADLAKYICENQDSISSKLKECCEKPLLEKSHCIAEVENDEMPADLPSLAADFVESKDVCKNYAEAKDVFLGMFLYEYARRHPDYSVVLLLRLAKTYETTLEKCCAAADPHECYAKVFDEFKPLVEEPQNLIKQNCELFEQLGEYKFQNALLVRYTKKVPQVSTPTLVEVSRNLGKVGSKCCKHPEAKRMPCVEDYLSVVLNQLCVLHEKTPVSDRVTKCCTESLVNRRPCFSALEVDETYVPKEFNAETFTFHADICTLSEKERQIKKQTALVELVKHKPKATKEQLKAVMDDFAAFVEKCCKADDKETCFAEEGKKLVAASQAALGL

SEQ ID NO: 86 - protein, 585 aa, Artificial Sequence
  HSA variant
DAHKSEVAHRFKDLGEENFKALVLIAFAQYLQQCPFEDHVKLVNEVTEFAKTCVADESAENCDKSLHTLFGDKLCTVATLRETYGEMADCCAKQEPERNECFLQHKDDNPNLPRLVRPEVDVMCTAFHDNEETFLKKYLYEIARRHPYFYAPELLFFAKRYKAAFTECCQAADKAACLLPKLDELRDEGKASSAKQRLKCASLQKFGERAFKAWAVARLSQRFPKAEFAEVSKLVTDLTKVHTECCHGDLLECADDRADLAKYICENQDSISSKLKECCEKPLLEKSHCIAEVENDEMPADLPSLAADFVESKDVCKNYAEAKDVFLGMFLYEYARRHPDYSVVLLLRLAKTYETTLEKCCAAADPHECYAKVFDEFKPLVEEPQNLIKQNCELFEQLGEYKFQNALLVRYTKKVPQVSTPTLVEVSRNLGKVGSKCCKHPEAKRMPCAEDYLSVVLNQLCVLHEKMPVSDRVTKCCTESLVNRRPCFSALEVDETYVPKEFNAETFTFHADICTLSEKERQIKKQTALVELVKHKPKATKEQLKAVMDDFAAFVEKCCKADDKETCFAEEGKKLVAASQAALGL

SEQ ID NO: 87 - protein, 585 aa, Artificial Sequence
  HSA variant
DAHKSEVAHRFKDLGEENFKALVLIAFAQYLQQCPFEDHVKLVNEVTEFAKTCVADESAENCDKSLHTLFGDKLCTVATLRETYGEMADCCAKQEPERNECFLQHKDDNPNLPRLVRPEVDVMCTAFHDNEETFLKKYLYEIARRHPYFYAPELLFFAKRYKAAFTECCQAADKAACLLPKLDELRDEGKASSAKQRLKCASLQKFGERAFKAWAVARLSQRFPKAEFAEVSKLVTDLTKVHTECCHGDLLECADDRADLAKYICENQDSISSKLKECCEKPLLEKSHCIAEVENDEMPADLPSLAADFVESKDVCKNYAEAKDVFLGMFLYEYARRHPDYSVVLLLRLAKTYETTLEKCCAAADPHECYAKVFDEFKPLVEEPQNLIKQNCELFEQLGEYKFQNALLVRYTKKVPQVSTPTLVEVSRNLGKVGSKCCKHPEAKRMPCAEDYLSVVLNQLCVLHEKTPVSDRVTKCCTESLVNRRPCFSALEVDETYVPKEFNAETFTFHADICTLSEKERQIKKQTALVELVKHKPKATKEQLKAVMDDFTAFVEKCCKADDKETCFAEEGKKLVAASQAALGL

SEQ ID NO: 88 - protein, 60 aa, Artificial Sequence
  albumin binding domain (ABD) variant
MRGSHHHHHHGCLAEAKVLANRELDKYGVSDFYKRLINKAKTVEGVEALKLHILAALPQA

SEQ ID NO: 89 - DNA, 99 bp, Artificial Sequence
  nucleic acid sequence encoding GLP1 variant
atgcatggcgaaggcacctttaccagcgatgtgagtagctatctggaaggtcaggcggccaaagaatttattgcctggctggtgcgggggcgttagtaa

SEQ ID NO: 90 - DNA, 579 bp, Artificial Sequence
  nucleic acid sequence encoding hGH variant
atgtttccaaccattccactgtctcgcctgtttgataatgcaatgctgcgtgcacatcgtctgcatcagctggcatttgatacctatcaggaatttgaagaagcatatattccaaaagaacagaaatattctttcctgcaaaatccacagacctcttagtgtttttctgaatctattccaaccccatccaatcgtgaagagacccaacagaaatctaatctggaactgctgcgtatctctctgttactgattcagtcttggctggaaccagtgcagttcctgcgttctgtgttcgcaaattctctggtttatggtgcatctgattctaatgtttatgatctgctgaaagatttagaggaaggaattcagaccctgatgggtcgtctggaagatggttctccacgtaccggtcagatttttaaacagacctattctaaatttgataccaattctcataatgacgatgcactgctgaaaaactatggtctgctgtactgctttcgtaaagatatggataaagttgaaacctttctgcgtattgttcagtgtcgttctgttgaaggttcttgtggtttttaa

SEQ ID NO: 91 - DNA, 579 bp, Artificial Sequence
  nucleic acid sequence encoding hGH variant
atgtttccaaccattccactgtctcgcctgtttgataatgcaatgctgcgtgcacatcgtctgcatcagctggcatttgatacctatcaggaatttgaagaagcatatattccaaaagaacagaaatattctttcctgcaaaatccacagacctctctgtgtttttctgaatctattccaaccccatccaatcgtgaagagacccaacagaaatctaatctggaactgctgcgtatctctctgttactgattcagtcttggctggaaccagtgcagttcctgcgttctgtgttcgcaaattctctggtttatggtgcatctgattctaatgtttatgatctgctgaaagatttagaggaaggaattcagaccctgatgggtcgtctggaagatggttctccacgtaccggtcagatttttaaatagacctattctaaatttgataccaattctcataatgacgatgcactgctgaaaaactatggtctgctgtactgctttcgtaaagatatggataaagttgaaacctttctgcgtattgttcagtgtcgttctgttgaaggttcttgtggtttttaa

SEQ ID NO: 92 - DNA, 720 bp, Artificial Sequence
  nucleic acid sequence encoding sfGFP variant
atgggatctatgagtaaaggagaagaacttttcactggagttgtcccaattcttgttgaattagatggtgatgttaatgggcacaaattttctgtccgtggagagggtgaaggtgatgcaacaaacggaaaacttacccttaaatttatttgcactactggaaaactacctgttccatggccaacacttgtcactactctgacctatggtgttcaatgcttctcccgttatccggatcatatgaaacggcatgactttttcaagagtgccatgcccgaaggttatgtacaggaacgcactataagcttcaaagatgacgggacctacaagacgcgtgctgaagtcaagtttgaaggtgatacccttgttaatcgtatcgagttaaaaggtattgattttaaagaagatggaaacattctcggacacaaactcgagtacaactttaactcacactaggtatacatcaccgcagacaaacaaaagaatggaatcaaagctaacttcaaaattcgccacaacgttgaagatggatccgttcaactagcagaccattatcaacaaaatactccaattggcgatggccctgtccttttaccagacaaccattacctgtcgacacaatctgtcctttcgaaagatcccaacgaaaagcgtgaccacatggtccttcttgagtttgtaactgctgctgggattacacatggcatggatgagctctaa

SEQ ID NO: 93 - DNA, 40 bp, Artificial Sequence
  primer
aaggcacctttaccagcgattagagtagctatctggaagg

SEQ ID NO: 94 - DNA, 40 bp, Artificial Sequence
  primer
ccttccagatagctactctaatcgctggtaaaggtgcctt

SEQ ID NO: 95 - DNA, 31 bp, Artificial Sequence
  primer
gcgatgtgagtagctagctggaaggtcaggc

SEQ ID NO: 96 - DNA, 31 bp, Artificial Sequence
  primer
gcctgaccttccagctagctactcacatcgc

SEQ ID NO: 97 - DNA, 36 bp, Artificial Sequence
  primer
gtcaggcggccaaagaatagattgcctggctggtgc

SEQ ID NO: 98 - DNA, 36 bp, Artificial Sequence
  primer
gcaccagccaggcaatctattctttggccgcctgac

SEQ ID NO: 99 - DNA, 30 bp, Artificial Sequence
  primer
gtgcgggggcgttagtaaggtaccatatgg

SEQ ID NO: 100 - DNA, 30 bp, Artificial Sequence
  primer
ccatatggtaccttactaacgcccccgcac

SEQ ID NO: 101 - DNA, 37 bp, Artificial Sequence
  primer
gcatcgaaggtaggcatggtgaaggcacctttaccag

SEQ ID NO: 102 - DNA, 37 bp, Artificial Sequence
  primer
ctggtaaaggtgccttcaccatgcctaccttcgatgc

SEQ ID NO: 103 - DNA, 33 bp, Artificial Sequence
  primer
ctgcaggtcgacttactaacgcccccgcaccag

SEQ ID NO: 104 - DNA, 33 bp, Artificial Sequence
  primer
ctggtgcgggggcgttagtaagtcgacctgcag

SEQ ID NO: 105 - DNA, 47 bp, Artificial Sequence
  primer
gttctccacgtaccggtcagatttttaaatagacctattctaaattt

SEQ ID NO: 106 - DNA, 47 bp, Artificial Sequence
  primer
aaatttagaataggtctatttaaaaatctgaccggtacgtggagaac

SEQ ID NO: 107 - DNA, 25 bp, Artificial Sequence
  primer
gccgccatggtgtctgctgtgaagg

SEQ ID NO: 108 - DNA, 25 bp, Artificial Sequence
  primer
gccgagatctttaatggtgatggtg

SEQ ID NO: 109 - DNA, 37 bp, Artificial Sequence
  primer
gtcgaagtccacctatacggtgttgtaacgccaacgg

SEQ ID NO: 110 - DNA, 37 bp, Artificial Sequence
  primer
ccgttggcgttacaacaccgtataggtggacttcgac

SEQ ID NO: 111 - protein, 16 aa, Artificial Sequence
  AgUox-WT fragment
YNTVEVDFDAVYASVR

SEQ ID NO: 112 - protein, 16 aa, Artificial Sequence
  AgUox variant fragment
  MISC_FEATURE (1)..(16): X is unnatural amino acid comprising tetrazine group or its variant, or triazine group or its variant.
YNTVXVDFDAVYASVR

SEQ ID NO: 113 - protein, 19 aa, Artificial Sequence
  AgUox variant fragment
AVIETHPEIDEIKMSLPNK